European Patent Application EP 4 502 150 A1, published February 5, 2025. Title: ENGINEERED IMMUNE CELL WITH CD7 GENE KNOCK-OUT AND USE THEREOF. Applicant: NANJING BIOHENG BIOTECH CO., LTD. Application EP. The sequence listing filed with the application follows.

SEQUENCE LISTING (26 sequences)

SEQ ID NO: 1 - RNA, 20 nt, synthetic construct
  source 1..20: mol_type = other RNA; note = 7-1
gtcacggaggtcaatgtcta

SEQ ID NO: 2 - RNA, 20 nt, synthetic construct
  source 1..20: mol_type = other RNA; note = 7-2
gtagacattgacctccgtga

SEQ ID NO: 3 - RNA, 20 nt, synthetic construct
  source 1..20: mol_type = other RNA; note = 7-3
gaggtcaatgtctacggctc

SEQ ID NO: 4 - RNA, 20 nt, synthetic construct
  source 1..20: mol_type = other RNA; note = 7-4
ggttgacggaggctcccacg

SEQ ID NO: 5 - RNA, 20 nt, synthetic construct
  source 1..20: mol_type = other RNA; note = 7-5
ggtacggacagacggttccg

SEQ ID NO: 6 - RNA, 20 nt, synthetic construct
  source 1..20: mol_type = other RNA; note = 7-6
gggaccctgagaagtcgatg

SEQ ID NO: 7 - RNA, 20 nt, synthetic construct
  source 1..20: mol_type = other RNA; note = 7-7
ggagcaggtgatgttgacgg

SEQ ID NO: 8 - RNA, 20 nt, synthetic construct
  source 1..20: mol_type = other RNA; note = 7-8
gtggcgggataagaattcgg

SEQ ID NO: 9 - RNA, 20 nt, synthetic construct
  source 1..20: mol_type = other RNA; note = 7-9
gtagacattgacctccgtga

SEQ ID NO: 10 - RNA, 20 nt, synthetic construct
  source 1..20: mol_type = other RNA; note = 7-10
ggagcaggtgatgttgacgg

SEQ ID NO: 11 - RNA, 20 nt, synthetic construct
  source 1..20: mol_type = other RNA; note = TRAC sgRNA
agagtctctcagctggtaca

SEQ ID NO: 12 - protein, 108 aa, synthetic construct
  source 1..108: note = anti-CD7 VL
DIELTQSPATLSVTPGDSVSLSCRASQSISNNLHWYQQKSHESPRLLIKSASQSISGIPSRFSGSGSGTDFTLSINSVETEDFGMYFCQQSNSWPYTFGGGTKLEIKR

SEQ ID NO: 13 - protein, 123 aa, synthetic construct
  source 1..123: note = anti-CD7 VH
QVQLQESGAELVKPGASVKLSCKASGYTFTSYWMHWVKQRPGQGLEWIGKINPSNGRTNYNEKFKSKATLTVDKSSSTAYMQLSSLTSEDSAVYYCARGGVYYDLYYYALDYWGQGTTVTVSS

SEQ ID NO: 14 - protein, 249 aa, synthetic construct
  source 1..249: note = anti-CD7 scFv
DIELTQSPATLSVTPGDSVSLSCRASQSISNNLHWYQQKSHESPRLLIKSASQSISGIPSRFSGSGSGTDFTLSINSVETEDFGMYFCQQSNSWPYTFGGGTKLEIKRGSTSGSGKPGSGEGSTKGQVQLQESGAELVKPGASVKLSCKASGYTFTSYWMHWVKQRPGQGLEWIGKINPSNGRTNYNEKFKSKATLTVDKSSSTAYMQLSSLTSEDSAVYYCARGGVYYDLYYYALDYWGQGTTVTVSS

SEQ ID NO: 15 - protein, 25 aa, synthetic construct
  source 1..25: note = CD8alpha transmembrane domain
IYIWAPLAGTCGVLLLSLVITLYCK

SEQ ID NO: 16 - DNA, 75 bp, synthetic construct
  source 1..75: mol_type = other DNA; note = CD8alpha transmembrane domain
atctacatctgggcgcccttggccgggacttgtggggtccttctcctgtcactggttatcaccctttactgcaaa

SEQ ID NO: 17 - protein, 45 aa, synthetic construct
  source 1..45: note = CD8alpha hinge region
TTTPAPRPPTPAPTIASQPLSLRPEACRPAAGGAVHTRGLDFACD

SEQ ID NO: 18 - DNA, 135 bp, synthetic construct
  source 1..135: mol_type = other DNA; note = CD8alpha hinge region
accacgacgccagcgccgcgaccaccaacaccggcgcccaccatcgcgtcgcagcccctgtccctgcgcccagaggcgtgccggccagcggcggggggcgcagtgcacacgagggggctggacttcgcctgtgat

SEQ ID NO: 19 - protein, 113 aa, synthetic construct
  source 1..113: note = CD3zeta primary signaling domain
LRVKFSRSADAPAYQQGQNQLYNELNLGRREEYDVLDKRRGRDPEMGGKPRRKNPQEGLYNELQKDKMAEAYSEIGMKGERRRGKGHDGLYQGLSTATKDTYDALHMQALPPR

SEQ ID NO: 20 - DNA, 339 bp, synthetic construct
  source 1..339: mol_type = other DNA; note = CD3zeta primary signaling domain
ctgagagtgaagttcagcaggagcgcagacgcccccgcgtaccagcagggccagaaccagctctataacgagctcaatctaggacgaagagaggagtacgatgttttggacaagagacgtggccgggaccctgagatggggggaaagccgagaaggaagaaccctcaggaaggcctgtacaatgaactgcagaaagataagatggcggaggcctacagtgagattgggatgaaaggcgagcgccggaggggcaaggggcacgatggcctttaccagggtctcagtacagccaccaaggacacctacgacgcccttcacatgcaggccctgccccctcgc

SEQ ID NO: 21 - protein, 114 aa, synthetic construct
  source 1..114: note = CD3zeta primary signaling domain
LRVKFSRSADAPAYQQGQNQLFNELNLGRREEFDVLDKRRGRDPEMGGKPQRRKNPQEGLYNELQKDKMAEAYSEIGMKGERRRGKGHDGLFQGLSTATKDTFDALHMQALPPR

SEQ ID NO: 22 - DNA, 342 bp, synthetic construct
  source 1..342: mol_type = other DNA; note = CD3zeta primary signaling domain
ctgagagtgaagttcagcaggagcgcagacgcccccgcgtaccagcagggccagaaccagctctttaacgagctcaatctaggacgaagagaggagttcgatgttttggacaagagacgtggccgggaccctgagatggggggaaagccgcagagaaggaagaaccctcaggaaggcctgtacaatgaactgcagaaagataagatggcggaggcctacagtgagattgggatgaaaggcgagcgccggaggggcaaggggcacgatggccttttccagggtctcagtacagccaccaaggacacctttgacgcccttcacatgcaggccctgccccctcgc

SEQ ID NO: 23 - protein, 40 aa, synthetic construct
  source 1..40: note = 4-1BB costimulatory domain
RGRKKLLYIFKQPFMRPVQTTQEEDGCSCRFPEEEEGGCE

SEQ ID NO: 24 - DNA, 120 bp, synthetic construct
  source 1..120: mol_type = other DNA; note = 4-1BB costimulatory domain
cggggcagaaagaaactcctgtatatattcaaacaaccatttatgagaccagtacaaactactcaagaggaagatggctgtagctgccgatttccagaagaagaagaaggaggatgtgaa

SEQ ID NO: 25 - protein, 21 aa, synthetic construct
  source 1..21: note = CD8alpha signal peptide
MALPVTALLLPLALLLHAARP

SEQ ID NO: 26 - DNA, 63 bp, synthetic construct
  source 1..63: mol_type = other DNA; note = CD8alpha signal peptide
atggccttaccagtgaccgccttgctcctgccgctggccttgctgctccacgccgccaggccg